European Patent Application EP 4 813 198 A1, published September 30, 2026. Title: J3 chaperone for increasing chromosomal recombination in meiosis of plant and uses thereof. Applicant: POSTECH Research and Business Development Foundation. Application KR. The sequence listing filed with the application follows.

SEQUENCE LISTING (36 sequences)

SEQ ID NO: 1 - DNA, 2403 bp, Arabidopsis thaliana
  source 1..2403: mol_type = genomic DNA
tctagagagttccaaactccacaaaacctcaaacaaaagcaaacgcaatttagcctcttcataagagagaagtcctctcagagaaacggcagccacatcaaccaacccaaacatcgaaagagagacacttttctctctctctttctctatctccttccaatctctctagggttttcgttacaacggcgaaaagatgttcggtagaggaccctcgaagaagagcgacaacactaagttctacgagatcttaggtgttcctaagagcgcttcaccagaagatctcaagaaagcttacaaaaaagccgctatcaagaatcatcctgataagggtggagatcccgagaaggtgaataatttcttagatccgcttagattctctcgaattcgattgtttgattgtgttttttttttcgattgatttgttgtcttgttagtttcttaatgttgaattttgatccgatctgataaaaaagtttgagttttggcgattaatcaaaaattagggttttgatgatatagatgtgtcttgctttgataattgagtggttaaagtttggttctttgttaggttatgagtttgatttgttgtgttatgtgttgattgcagtttaaggagttagcacaagcttatgaagtgcttagtgacccggagaagcgtgagatttatgaccagtatggagaggatgcactcaaggaaggaatgggtggtggaggaggtggacatgatccatttgatattttctcatccttctttggtggaggcccctttggaggtgagtctccttggacactgtacactttatgatatcgcaattgagaattttcgtttgaatatgtttctgtttttgaataggtaataccagccggcaaaggaggcagaggcgtggtgaggatgttgttcatcccttgaaggtatctcttgaggatgtgtaccttggtacaatgaagaagctttcactttctaggaatgctctctgctctaagtgtaacgggttagtacattcgactcgatcttgcgtttttggtgtagctatatgtgtcctaggttcataataatatgaattagcttaagttttgacagaaaccctttatctcaatttgtgaccccagttggttaaaaggttctgaatttgtgattgcagaaagggatcaaaatctggagcctccttgaaatgtggagggtgtcagggatctggtatgaaggtgtctattaggcagcttggacctggaatgatccagcagatgcagcatgcatgtaatgaatgcaaagggacaggtgagaccatcaatgatcgggacaggtgtccacaatgcaaaggagacaaggtcattcctgagaagaaggtgcttgaagtgaatgtggagaagggaatgcaacacagtcagaagatcacatttgaaggacaagcagatgaagcggtatctactctcatacatttactccagctttgattactagtatgtttacttttcttctggagactaaccttttgttttatgttttggtgttggtgcagcctgacactgtcactggagatatagtgtttgtccttcagcagaaagagcacccaaagttcaagagaaagggagaagacctctttgtggagcacacactttctctaaccgaagctttgtgtggcttccaatttgttctgactcacttggatggcagaagtcttctcattaaatctaatcctggggaggtcgtgaaacctggtacgtattcagatgcatcgtcatactcagattttacagttactataactgtctctgattgaaacatgatcacttatcttatgtgtttgacagattcatacaaggcaataagcgatgaaggaatgccgatataccagaggccattcatgaagggtaagctctacatccacttcacagtggagttcccggactcgttgagcccagatcagaccaaagcactggaagctgttctacctaagccgtcaacagctcagttgagtgacatggagatagatgaatgcgaggagaccacgctccacgatgtcaacattgaggatgagatgaggaggaaggcacaagctcaaagagaggcttatgatgatgacgatgaagatgatgaccatccgggtggtgctcaaagggtgcaatgtgcccagcagtaagtaactccttagagagactttgacccacatgggtttgggctccaaccaatttgtctcttgctttttcattctaagtgtattggagtctttatgggagtttggtacggtttaagaatttgcccacttcggtggaacatcgaaacttgttttctctttttcctctgactttaaaaattaaggccttattacaattttgtgttttttctttatgattaaatttgtagtaatttaatgtctaagaacatatatactgtgtgttttctat

SEQ ID NO: 2 - DNA, 1263 bp, Arabidopsis thaliana
  source 1..1263: mol_type = genomic DNA
atgttcggtagaggaccctcgaagaagagcgacaacactaagttctacgagatcttaggtgttcctaagagcgcttcaccagaagatctcaagaaagcttacaaaaaagccgctatcaagaatcatcctgataagggtggagatcccgagaagtttaaggagttagcacaagcttatgaagtgcttagtgacccggagaagcgtgagatttatgaccagtatggagaggatgcactcaaggaaggaatgggtggtggaggaggtggacatgatccatttgatattttctcatccttctttggtggaggcccctttggaggtaataccagccggcaaaggaggcagaggcgtggtgaggatgttgttcatcccttgaaggtatctcttgaggatgtgtaccttggtacaatgaagaagctttcactttctaggaatgctctctgctctaagtgtaacggaaagggatcaaaatctggagcctccttgaaatgtggagggtgtcagggatctggtatgaaggtgtctattaggcagcttggacctggaatgatccagcagatgcagcatgcatgtaatgaatgcaaagggacaggtgagaccatcaatgatcgggacaggtgtccacaatgcaaaggagacaaggtcattcctgagaagaaggtgcttgaagtgaatgtggagaagggaatgcaacacagtcagaagatcacatttgaaggacaagcagatgaagcgcctgacactgtcactggagatatagtgtttgtccttcagcagaaagagcacccaaagttcaagagaaagggagaagacctctttgtggagcacacactttctctaaccgaagctttgtgtggcttccaatttgttctgactcacttggatggcagaagtcttctcattaaatctaatcctggggaggtcgtgaaacctgattcatacaaggcaataagcgatgaaggaatgccgatataccagaggccattcatgaagggtaagctctacatccacttcacagtggagttcccggactcgttgagcccagatcagaccaaagcactggaagctgttctacctaagccgtcaacagctcagttgagtgacatggagatagatgaatgcgaggagaccacgctccacgatgtcaacattgaggatgagatgaggaggaaggcacaagctcaaagagaggcttatgatgatgacgatgaagatgatgaccatccgggtggtgctcaaagggtgcaatgtgcccagcagtaa

SEQ ID NO: 3 - protein, 420 aa, Arabidopsis thaliana
MFGRGPSKKSDNTKFYEILGVPKSASPEDLKKAYKKAAIKNHPDKGGDPEKFKELAQAYEVLSDPEKREIYDQYGEDALKEGMGGGGGGHDPFDIFSSFFGGGPFGGNTSRQRRQRRGEDVVHPLKVSLEDVYLGTMKKLSLSRNALCSKCNGKGSKSGASLKCGGCQGSGMKVSIRQLGPGMIQQMQHACNECKGTGETINDRDRCPQCKGDKVIPEKKVLEVNVEKGMQHSQKITFEGQADEAPDTVTGDIVFVLQQKEHPKFKRKGEDLFVEHTLSLTEALCGFQFVLTHLDGRSLLIKSNPGEVVKPDSYKAISDEGMPIYQRPFMKGKLYIHFTVEFPDSLSPDQTKALEAVLPKPSTAQLSDMEIDECEETTLHDVNIEDEMRRKAQAQREAYDDDDEDDDHPGGAQRVQCAQQ

SEQ ID NO: 4 - DNA, 30 bp, synthetic construct
  source 1..30: mol_type = other DNA
cacatttcaaggaggctccagatttggatc

SEQ ID NO: 5 - DNA, 22 bp, synthetic construct
  source 1..22: mol_type = other DNA
gctatatgtgtcctaggttcat

SEQ ID NO: 6 - DNA, 19 bp, synthetic construct
  source 1..19: mol_type = other DNA
attttgccgatttcggaac

SEQ ID NO: 7 - DNA, 22 bp, synthetic construct
  source 1..22: mol_type = other DNA
tgttgaattttgatccgatctg

SEQ ID NO: 8 - DNA, 21 bp, synthetic construct
  source 1..21: mol_type = other DNA
ccctttctcttgaactttggg

SEQ ID NO: 9 - DNA, 47 bp, synthetic construct
  source 1..47: mol_type = other DNA
gcctgcaggtcgactctagagaaatcagtgatgatcaaattacttac

SEQ ID NO: 10 - DNA, 45 bp, synthetic construct
  source 1..45: mol_type = other DNA
aggcgcgccctcgagttgaactctttttaaaatacaactggtatg

SEQ ID NO: 11 - DNA, 54 bp, synthetic construct
  source 1..54: mol_type = other DNA
ccgaagacggctcaggagccaacctacttgcatgttaacaagaaactattattc

SEQ ID NO: 12 - DNA, 41 bp, synthetic construct
  source 1..41: mol_type = other DNA
ccgaagacggctcgatggcttttcgccgttgtaacgaaaac

SEQ ID NO: 13 - DNA, 39 bp, synthetic construct
  source 1..39: mol_type = other DNA
aaagaagacaactcaaatgatgttcggtagaggaccctc

SEQ ID NO: 14 - DNA, 34 bp, synthetic construct
  source 1..34: mol_type = other DNA
aaagaagacaaacctttactgctgggcacattgc

SEQ ID NO: 15 - DNA, 29 bp, synthetic construct
  source 1..29: mol_type = other DNA
attgcagaaagagatcaaaatctggagcc

SEQ ID NO: 16 - DNA, 29 bp, synthetic construct
  source 1..29: mol_type = other DNA
ggctccagattttgatctctttctgcaat

SEQ ID NO: 17 - DNA, 42 bp, synthetic construct
  source 1..42: mol_type = other DNA
ccgaagacggctcagcttgtaactccttagagagactttgac

SEQ ID NO: 18 - DNA, 45 bp, synthetic construct
  source 1..45: mol_type = other DNA
ccgaagacggctcgagcgaactctttttaaaatacaactggtatg

SEQ ID NO: 19 - DNA, 43 bp, synthetic construct
  source 1..43: mol_type = other DNA
ccgaagacggctcaggagaaagaaaccaaagttccatgtccat

SEQ ID NO: 20 - DNA, 45 bp, synthetic construct
  source 1..45: mol_type = other DNA
ccgaagacggctcgcattccgatcactgacacaagcaaaaataaa

SEQ ID NO: 21 - DNA, 41 bp, synthetic construct
  source 1..41: mol_type = other DNA
cccgaagacggctcaaatgatgagatgcaacgcgtgttgga

SEQ ID NO: 22 - DNA, 45 bp, synthetic construct
  source 1..45: mol_type = other DNA
ccgaagacggctcgcgaacctagcgtgaacagctgagggcgggaa

SEQ ID NO: 23 - DNA, 40 bp, synthetic construct
  source 1..40: mol_type = other DNA
ccgaagacggctcaaatgatggaggaaatggaggacactg

SEQ ID NO: 24 - DNA, 42 bp, synthetic construct
  source 1..42: mol_type = other DNA
ccgaagacggctcgcgaaccggaagtgaagatatcttgaaag

SEQ ID NO: 25 - DNA, 36 bp, synthetic construct
  source 1..36: mol_type = other DNA
ccgaagacggctcaaatgatggcgacggcgggatca

SEQ ID NO: 26 - DNA, 41 bp, synthetic construct
  source 1..41: mol_type = other DNA
ccgaagacggctcgcgaacctcagttgaatttgggactgag

SEQ ID NO: 27 - DNA, 48 bp, synthetic construct
  source 1..48: mol_type = other DNA
ccgaagacggctcaggagccataatcgtgagtagatatattactcaac

SEQ ID NO: 28 - DNA, 49 bp, synthetic construct
  source 1..49: mol_type = other DNA
ccgaagacggctcgcattggctgtggtgagagaaacagagcgtgagctc

SEQ ID NO: 29 - DNA, 41 bp, synthetic construct
  source 1..41: mol_type = other DNA
cccgaagacggctcaggagatggaggtagcgggataattga

SEQ ID NO: 30 - DNA, 58 bp, synthetic construct
  source 1..58: mol_type = other DNA
cccgaagacggctcgcattcccgcgtgcaatgtagcggccatccttaagaagaagaaa

SEQ ID NO: 31 - DNA, 39 bp, synthetic construct
  source 1..39: mol_type = other DNA
cccgaagacggctcaggagtggcaggatatattgtggtg

SEQ ID NO: 32 - DNA, 42 bp, synthetic construct
  source 1..42: mol_type = other DNA
cccgaagacggctcgcattccttttgcagaagtgtgaaacga

SEQ ID NO: 33 - DNA, 40 bp, synthetic construct
  source 1..40: mol_type = other DNA
cccgaagacggctcaggaggacctctctgttcttaattcc

SEQ ID NO: 34 - DNA, 45 bp, synthetic construct
  source 1..45: mol_type = other DNA
cccgaagacggctcgcattccctctttcgagtttcaaaactgaaa

SEQ ID NO: 35 - DNA, 39 bp, synthetic construct; identical to SEQ ID NO: 31
  source 1..39: mol_type = other DNA

SEQ ID NO: 36 - DNA, 46 bp, synthetic construct
  source 1..46: mol_type = other DNA
cccgaagacggctcgcattcctttttctccgtacgaaagcttgaaa